European Patent Specification EP 2 760 887 B1, published October 23, 2024. Title: Compositions and Methods for Modulating Hemostasis. Applicant: Camire, Rodney M. Application PCT/US2012/058279. The sequence listing filed with the application follows.

SEQUENCE LISTING (7 sequences)

SEQ ID NO: 1 - protein, 4 aa, Artificial Sequence
  Synthetic Sequence
IVGG

SEQ ID NO: 2 - protein, 488 aa, Homo sapiens
MGRPLHLVLLSASLAGLLLLGESLFIRREQANNILARVRRANSFLEEMKKGHLERECMEETCSYEEAREVFEDSDKTNEFWNKYKDGDQCETSPCQNQGKCKDGLGEYTCTCLEGFEGKNCELFTRKLCSLDNGDCDQFCHEEQNSVVCSCARGYTLADNGKACIPTGPYPCGKQTLERRKRSVAQATSSSGEAPDSITWKPYDAADLDPTENPFDLLDFNQTQPERGDNNLTRIVGGQECKDGECPWQALLINEENEGFCGGTILSEFYILTAAHCLYQAKRFKVRVGDRNTEQEEGGEAVHEVEVVIKHNRFTKETYDFDIAVLRLKTPITFRMNVAPACLPERDWAESTLMTQKTGIVSGFGRTHEKGRQSTRLKMLEVPYVDRNSCKLSSSFIITQNMFCAGYDTKQEDACQGDSGGPHVTRFKDTYFVTGIVSWGEGCARKGKYGIYTKVTAFLKWIDRSMKTRGLPKAKSHAPEVITSSPLK

SEQ ID NO: 3 - protein, 139 aa, Homo sapiens
ANSFLEEMKKGHLERECMEETCSYEEAREVFEDSDKTNEFWNKYKDGDQCETSPCQNQGKCKDGLGEYTCTCLEGFEGKNCELFTRKLCSLDNGDCDQFCHEEQNSVVCSCARGYTLADNGKACIPTGPYPCGKQTLER

SEQ ID NO: 4 - protein, 306 aa, Homo sapiens
SVAQATSSSGEAPDSITWKPYDAADLDPTENPFDLLDFNQTQPERGDNNLTRIVGGQECKDGECPWQALLINEENEGFCGGTILSEFYILTAAHCLYQAKRFKVRVGDRNTEQEEGGEAVHEVEVVIKHNRFTKETYDFDIAVLRLKTPITFRMNVAPACLPERDWAESTLMTQKTGIVSGFGRTHEKGRQSTRLKMLEVPYVDRNSCKLSSSFIITQNMFCAGYDTKQEDACQGDSGGPHVTRFKDTYFVTGIVSWGEGCARKGKYGIYTKVTAFLKWIDRSMKTRGLPKAKSHAPEVITSSPLK

SEQ ID NO: 5 - protein, 254 aa, Homo sapiens [sequence omitted]

SEQ ID NO: 6 - DNA, 1467 bp, Homo sapiens
atggggcgcccactgcacctcgtcctgctcagtgcctccctggctggcctcctgctgctcggggaaagtctgttcatccgcagggagcaggccaacaacatcctggcgagggtcaggagggccaattcctttcttgaagagatgaagaaaggacacctcgaaagagagtgcatggaagagacctgctcatacgaagaggcccgcgaggtctttgaggacagcgacaagacgaatgaattctggaataaatacaaagatggcgaccagtgtgagaccagtccttgccagaaccagggcaaatgtaaagacggcctcggggaatacacctgcacctgtttagaaggattcgaaggcaaaaactgtgaattattcacacggaagctctgcagcctggacaacggggactgtgaccagttctgccacgaggaacagaactctgtggtgtgctcctgcgcccgcgggtacaccctggctgacaacggcaaggcctgcattcccacagggccctacccctgtgggaaacagaccctggaacgcaggaagaggtcagtggcccaggccaccagcagcagcggggaggcccctgacagcatcacatggaagccatatgatgcagccgacctggaccccaccgagaaccccttcgacctgcttgacttcaaccagacgcagcctgagaggggcgacaacaacctcacgcgtatcgtgggaggccaggaatgcaaggacggggagtgtccctggcaggccctgctcatcaatgaggaaaacgagggtttctgtggtggaactattctgagcgagttctacatcctaacggcagcccactgtctctaccaagccaagagattcaaggtgagggtaggtgaccggaacacggagcaggaggagggcggtgaggcggtgcacgaggtggaggtggtcatcaagcacaaccggttcacaaaggagacctatgacttcgacatcgccgtgctccggctcaagacccccatcaccttccgcatgaacgtggcgcctgcctgcctccccgagcgtgactgggccgagtccacgctgatgacgcagaagacggggattgtgagcggcttcgggcgcacccacgagaagggccggcagtccaccaggctcaagatgctggaggtgccctacgtggaccgcaacagctgcaagctgtccagcagcttcatcatcacccagaacatgttctgtgccggctacgacaccaagcaggaggatgcctgccagggggacagcgggggcccgcacgtcacccgcttcaaggacacctacttcgtgacaggcatcgtcagctggggagagggctgtgcccgtaaggggaagtacgggatctacaccaaggtcaccgccttcctcaagtggatcgacaggtccatgaaaaccaggggcttgcccaaggccaagagccatgccccggaggtcataacgtcctctccattaaagtga

SEQ ID NO: 7 - protein, 6 aa, Artificial Sequence
  proteolytic cleavage site
RKRRKR